European Patent Specification EP 4 259 652 B1, published February 19, 2025. Title: Assay for detecting Collagen XVIII biomarkers. Applicant: Nordic Bioscience A/S. The sequence listing filed with the application follows.

SEQUENCE LISTING (20 sequences)

SEQ ID NO: 1 - protein, 6 aa, Artificial Sequence
  Synthetic peptide
NLLNLN

SEQ ID NO: 2 - protein, 10 aa, Artificial Sequence
  Synthetic peptide
NLLNLNKDKE

SEQ ID NO: 3 - protein, 5 aa, Artificial Sequence
  Synthetic peptide
DYWIH

SEQ ID NO: 4 - protein, 17 aa, Artificial Sequence
  Synthetic peptide
EINPSDGRSNYNEKFKT

SEQ ID NO: 5 - protein, 6 aa, Artificial Sequence
  Synthetic peptide
DLGFAD

SEQ ID NO: 6 - protein, 16 aa, Artificial Sequence
  Synthetic peptide
RSSQSIVYSNGNTYLQ

SEQ ID NO: 7 - protein, 7 aa, Artificial Sequence
  Synthetic peptide
KVSNRFS

SEQ ID NO: 8 - protein, 9 aa, Artificial Sequence
  Synthetic peptide
FQGSHVPFT

SEQ ID NO: 9 - protein, 89 aa, Artificial Sequence
  Synthetic peptide
RSSQSIVYSNGNTYLQWYLQKPGQSPQLLIYKVSNRFSGVPDRFSGSGSGTDFTLKISRVEAEDVGVYYCFQGSHVPFTFGSGTKLEIK

SEQ ID NO: 10 - protein, 85 aa, Artificial Sequence
  Synthetic peptide
DYWIHWVKQRPGQGLEWIGEINPSDGRSNYNEKFKTKATLTVDRSSSTAYMHLSSLTSEDSAVFYCARDLGFADWGPGTTVTVSS

SEQ ID NO: 11 - protein, 112 aa, Artificial Sequence
  Synthetic peptide
DILMTQTPLSLPVGLGDQASISCRSSQSIVYSNGNTYLQWYLQKPGQSPQLLIYKVSNRFSGVPDRFSGSGSGTDFTLKISRVEAEDVGVYYCFQGSHVPFTFGSGTKLEIK

SEQ ID NO: 12 - protein, 115 aa, Artificial Sequence
  Synthetic peptide
QVQLQQPGAELVKPGASVKLSCKASGYTFIDYWIHWVKQRPGQGLEWIGEINPSDGRSNYNEKFKTKATLTVDRSSSTAYMHLSSLTSEDSAVFYCARDLGFADWGPGTTVTVSS

SEQ ID NO: 13 - protein, 10 aa, Artificial Sequence
  Synthetic peptide
  MOD_RES 10: Amino acid is biotinylated via an optional linker
NLLNLNKDKE

SEQ ID NO: 14 - protein, 10 aa, Artificial Sequence
  Synthetic peptide
NLLNLNWLWF

SEQ ID NO: 15 - protein, 11 aa, Artificial Sequence
  Synthetic peptide
  MOD_RES 11: Biotinylated
NLLNLNKDKEK

SEQ ID NO: 16 - protein, 15 aa, Artificial Sequence
  Synthetic peptide
  MOD_RES 15: Bound to keyhole limpet hemocyanin
NLLNLNKDKEKKGGC

SEQ ID NO: 17 - protein, 10 aa, Artificial Sequence
  Synthetic peptide
LHDSNPYPRR

SEQ ID NO: 18 - protein, 10 aa, Artificial Sequence
  Synthetic peptide
NALNLNWLWF

SEQ ID NO: 19 - protein, 514 aa, Artificial Sequence
  Synthetic peptide
QVQLQQPGAELVKPGASVKLSCKASGYTFIDYWIHWVKQRPGQGLEWIGEINPSDGRSNYNEKFKTKATLTVDRSSSTAYMHLSSLTSEDSAVFYCARDLGFADWGPGTTVTVSSAKTTAPSVYPLAPVCGDTTGSSVTLGCLVKGYFPEPVTLTWNSGSLSSGVHTFPAVLQSDLYTLSSSVTVTSSTWPSQSITCNVAHPASSTKVDKKIEPRGPTIKPCPPCKCPAPNLLGGPSVFIFPPKIKDVLMISLSPIVTCVVVDVSEDDPDVQISWFVNNVEVHTAQTQTHREDYNSTLRVVSALPIQHQDWMSGKEFKCKVNNKDLPAPIERTISKPKGSVRAPQVYVLPPPEEEMTKKQVTLTCMVTDFMPEDIYVEWTNNGKTELNYKNTEPVLDSDGSYFMYSKLRVEKKNWVERNSYSCSVVHEGLHNHHTTKSFSRTPGLDLDDVCAEAQDGELDGLWTTITIFISLFLLSVCYSASVTLFKVKWIFSSVVELKQTISPDYRNMIGQGA

SEQ ID NO: 20 - protein, 219 aa, Artificial Sequence
  Synthetic peptide
DILMTQTPLSLPVGLGDQASISCRSSQSIVYSNGNTYLQWYLQKPGQSPQLLIYKVSNRFSGVPDRFSGSGSGTDFTLKISRVEAEDVGVYYCFQGSHVPFTFGSGTKLEIKRADAAPTVSIFPPSSEQLTSGGASVVCFLNNFYPKDINVKWKIDGSERQNGVLNSWTDQDSKDSTYSMSSTLTLTKDEYERHNSYTCEATHKTSTSPIVKSFNRNEC